European Patent Application EP 4 640 212 A1, published October 29, 2025. Title: FUNCTIONALIZED LIPOSOMAL COMPLEX, PHARMACEUTICAL COMPOSITION, COSMETIC COMPOSITION AND RELATED USES. Applicant: MARJAN IND E COMERCIO LTDA. Application BR WO2024130374, filed December 22, 2023. The sequence listing filed with the application follows.

SEQUENCE LISTING (9 sequences)

SEQ ID NO: 1 - DNA, 87 bp, synthetic construct
  source 1..87: mol_type = other DNA
atgagaagcgtcggtgtggttaaacacggaacgaaggtgcaggaagatttgtcgatgcggtgcctgagcgggctggcaaggcgcata

SEQ ID NO: 2 - DNA, 86 bp, synthetic construct
  source 1..86: mol_type = other DNA
atgagaagcgtcggtgtggttactccgggcacttgatatatcgatatggagaataatgcaccctgagcgggctggcaaggcgcata

SEQ ID NO: 3 - DNA, 40 bp, synthetic construct
  source 1..40: mol_type = other DNA
gttaccgcggtgaagggtggatgtgtctggacgctatatc

SEQ ID NO: 4 - DNA, 85 bp, synthetic construct
  source 1..85: mol_type = other DNA
atgagagcgtcggtgtggtannnnnnnnnnnnnnnnnnnnnnnnnnnnnnnnnnnnnnnnnnnnntacttccgcaccctcctaca

SEQ ID NO: 5 - DNA, 40 bp, synthetic construct
  source 1..40: mol_type = other DNA
gcccctagggggtgttcaacaggagtattatgatccttag

SEQ ID NO: 6 - DNA, 30 bp, synthetic construct
  source 1..30: mol_type = other DNA
cgactaactgttttcttttgtttttagtcg

SEQ ID NO: 7 - protein, 6 aa, unidentified
GGAGAA

SEQ ID NO: 8 - DNA, 17 bp, synthetic construct
  source 1..17: mol_type = other DNA
atacaactggattgtat

SEQ ID NO: 9 - DNA, 30 bp, synthetic construct
  source 1..30: mol_type = other DNA
acttttgaatgtggcaacaaattcgacagg